European Patent Application EP 4 659 764 A1, published December 10, 2025. Title: LINKER DRUG, AND PREPARATION METHOD AND USE OF ANTIBODY-DRUG CONJUGATE THEREOF. Applicant: SHANGHAI MIRACOGEN INC. The sequence listing filed with the application follows.

SEQUENCE LISTING (24 sequences)

SEQ ID NO: 1 - protein, 11 aa, synthetic construct
RASQDVNTAVA

SEQ ID NO: 2 - protein, 7 aa, synthetic construct
SASFLYS

SEQ ID NO: 3 - protein, 9 aa, synthetic construct
QQHYTTPPT

SEQ ID NO: 4 - protein, 10 aa, synthetic construct
GFNIKDTYIH

SEQ ID NO: 5 - protein, 17 aa, synthetic construct
RIYPTNGYTRYADSVKG

SEQ ID NO: 6 - protein, 11 aa, synthetic construct
WGGDGFYAMDY

SEQ ID NO: 7 - protein, 98 aa, synthetic construct
DIQMTQSPSSLSASVGDRVTITCRASQDVNTAVAWYQQKPGKAPKLLIYSASFLYSGVPSRFSGSRSGTDFTLTISSLQPEDFATYYCQQHYTTPPTF

SEQ ID NO: 8 - protein, 116 aa, synthetic construct
GQGTKVEIKRTVAAPSVFIFPPSDEQLKSGTASVVCLLNNFYPREAKVQWKVDNALQSGNSQESVTEQDSKDSTYSLSSTLTLSKADYEKHKVYACEVTHQGLSSPVTKSFNRGEC

SEQ ID NO: 9 - protein, 214 aa, synthetic construct
DIQMTQSPSSLSASVGDRVTITCRASQDVNTAVAWYQQKPGKAPKLLIYSASFLYSGVPSRFSGSRSGTDFTLTISSLQPEDFATYYCQQHYTTPPTFGQGTKVEIKRTVAAPSVFIFPPSDEQLKSGTASVVCLLNNFYPREAKVQWKVDNALQSGNSQESVTEQDSKDSTYSLSSTLTLSKADYEKHKVYACEVTHQGLSSPVTKSFNRGEC

SEQ ID NO: 10 - protein, 125 aa, synthetic construct
EVQLVESGGGLVQPGGSLRLSCAASGFNIKDTYIHWVRQAPGKGLEWVARIYPTNGYTRYADSVKGRFTISADTSKNTAYLQMNSLRAEDTAVYYCSRWGGDGFYAMDYWGQGTLVTVSSASTKG

SEQ ID NO: 11 - protein, 325 aa, synthetic construct
PSVFPLAPSSKSTSGGTAALGCLVKDYFPEPVTVSWNSGALTSGVHTFPAVLQSSGLYSLSSVVTVPSSSLGTQTYICNVNHKPSNTKVDKKVEPKSCDKTHTCPPCPAPELLGGPSVFLFPPKPKDTLMISRTPEVTCVVVDVSHEDPEVKFNWYVDGVEVHNAKTKPREEQYNSTYRVVSVLTVLHQDWLNGKEYKCKVSNKALPAPIEKTISKAKGQPREPQVYTLPPSREEMTKNQVSLTCLVKGFYPSDIAVEWESNGQPENNYKTTPPVLDSDGSFFLYSKLTVDKSRWQQGNVFSCSVMHEALHNHYTQKSLSLSPGK

SEQ ID NO: 12 - protein, 450 aa, synthetic construct
EVQLVESGGGLVQPGGSLRLSCAASGFNIKDTYIHWVRQAPGKGLEWVARIYPTNGYTRYADSVKGRFTISADTSKNTAYLQMNSLRAEDTAVYYCSRWGGDGFYAMDYWGQGTLVTVSSASTKGPSVFPLAPSSKSTSGGTAALGCLVKDYFPEPVTVSWNSGALTSGVHTFPAVLQSSGLYSLSSVVTVPSSSLGTQTYICNVNHKPSNTKVDKKVEPKSCDKTHTCPPCPAPELLGGPSVFLFPPKPKDTLMISRTPEVTCVVVDVSHEDPEVKFNWYVDGVEVHNAKTKPREEQYNSTYRVVSVLTVLHQDWLNGKEYKCKVSNKALPAPIEKTISKAKGQPREPQVYTLPPSREEMTKNQVSLTCLVKGFYPSDIAVEWESNGQPENNYKTTPPVLDSDGSFFLYSKLTVDKSRWQQGNVFSCSVMHEALHNHYTQKSLSLSPGK

SEQ ID NO: 13 - protein, 6 aa, synthetic construct
QSIGTN

SEQ ID NO: 14 - skipped

SEQ ID NO: 15 - protein, 9 aa, synthetic construct
QQNNEWPTS

SEQ ID NO: 16 - protein, 8 aa, synthetic construct
GFSLSNYD

SEQ ID NO: 17 - protein, 7 aa, synthetic construct
IWSGGNT

SEQ ID NO: 18 - protein, 13 aa, synthetic construct
ARALDYYDYEFAY

SEQ ID NO: 19 - protein, 70 aa, synthetic construct
EIVLTQSPDFQSVTPKEKVTITCRASQSIGTNIHWYQQKPDQSPKLLIKYASESISGIPSRFSGSGSGTD

SEQ ID NO: 20 - protein, 116 aa, synthetic construct
GQGTKLEIKRTVAAPSVFIFPPSDEQLKSGTASVVCLLNNFYPREAKVQWKVDNALQSGNSQESVTEQDSKDSTYSLSSTLTLSKADYEKHKVYACEVTHQGLSSPVTKSFNRGEC

SEQ ID NO: 21 - protein, 214 aa, synthetic construct
EIVLTQSPDFQSVTPKEKVTITCRASQSIGTNIHWYQQKPDQSPKLLIKYASESISGIPSRFSGSGSGTDFTLTINSLEAEDAATYYCQQNNEWPTSFGQGTKLEIKRTVAAPSVFIFPPSDEQLKSGTASVVCLLNNFYPREAKVQWKVDNALQSGNSQESVTEQDSKDSTYSLSSTLTLSKADYEKHKVYACEVTHQGLSSPVTKSFNRGEC

SEQ ID NO: 22 - protein, 109 aa, synthetic construct
QVQLQESGPGLVKPSETLSLTCTVSGFSLSNYDVHWVRQAPGKGLEWLGVIWSGGNTDYNTPFTSRLTISVDTSKNQFSLKLSSVTAADTAVYYCARALDYYDYEFAYW

SEQ ID NO: 23 - protein, 340 aa, synthetic construct
GQGTLVTVSSASTKGPSVFPLAPSSKSTSGGTAALGCLVKDYFPEPVTVSWNSGALTSGVHTFPAVLQSSGLYSLSSVVTVPSSSLGTQTYICNVNHKPSNTKVDKRVEPKSCDKTHTCPPCPAPELLGGPSVFLFPPKPKDTLMISRTPEVTCVVVDVSHEDPEVKFNWYVDGVEVHNAKTKPREEQYNSTYRVVSVLTVLHQDWLNGKEYKCKVSNKALPAPIEKTISKAKGQPREPQVYTLPPSREEMTKNQVSLTCLVKGFYPSDIAVEWESNGQPENNYKTTPPVLDSDGSFFLYSKLTVDKSRWQQGNVFSCSVMHEALHNHYTQKSLSLSPGK

SEQ ID NO: 24 - protein, 449 aa, synthetic construct
QVQLQESGPGLVKPSETLSLTCTVSGFSLSNYDVHWVRQAPGKGLEWLGVIWSGGNTDYNTPFTSRLTISVDTSKNQFSLKLSSVTAADTAVYYCARALDYYDYEFAYWGQGTLVTVSSASTKGPSVFPLAPSSKSTSGGTAALGCLVKDYFPEPVTVSWNSGALTSGVHTFPAVLQSSGLYSLSSVVTVPSSSLGTQTYICNVNHKPSNTKVDKRVEPKSCDKTHTCPPCPAPELLGGPSVFLFPPKPKDTLMISRTPEVTCVVVDVSHEDPEVKFNWYVDGVEVHNAKTKPREEQYNSTYRVVSVLTVLHQDWLNGKEYKCKVSNKALPAPIEKTISKAKGQPREPQVYTLPPSREEMTKNQVSLTCLVKGFYPSDIAVEWESNGQPENNYKTTPPVLDSDGSFFLYSKLTVDKSRWQQGNVFSCSVMHEALHNHYTQKSLSLSPGK